European Patent Application EP 4 218 811 A1, published August 2, 2023. Title: Method for treating a GD2 positive cancer. Applicant: Aperion Biologics AG. The sequence listing filed with the application follows.

SEQUENCE LISTING (8 sequences)

SEQ ID NO: 1 - DNA, 723 bp, synthetic construct
  source 1..723: mol_type = other DNA
  misc_feature 1..723: note = artificial antibody chain
atggaagccccagcgcagcttctcttcctcctgctactctggctcccagataccactggagaaatagtgatgacgcagtctccagccaccctgtctgtgtctccaggggaaagagccaccctctcctgcagatctagtcagagtcttgtacaccgtaatggaaacacctatttacattggtacctgcagaagccaggccagtctccaaagctcctgattcacaaagtttccaaccgattttctggggtcccagacaggttcagtggcagtggatcagggacagatttcacactcaagatcagcagagtggaggctgaggatctgggagtttatttctgttctcaaagtacacatgttcctccgctcacgttcggtgctgggaccaagctggagctgaaacgaactgtggctgcaccatctgtcttcatcttcccgccatctgatgagcagttgaaatctggaactgcctctgttgtgtgcctgctgaataacttctatcccagagaggccaaagtacagtggaaggtggataacgccctccaatcgggtaactcccaggagagtgtcacagagcaggacagcaaggacagcacctacagcctcagcagcaccctgacgctgagcaaagcagactacgagaaacacaaagtctacgcctgcgaagtcacccatcagggcctgagctcgcccgtcacaaagagcttcaacaggggagagtgttag

SEQ ID NO: 2 - DNA, 1389 bp, synthetic construct
  source 1..1389: mol_type = other DNA
  misc_feature 1..1389: note = artificial antibody chain
atgggatggacctggatctttattttaatcctgtcggtaactacaggtgtccactctgaggtccaactgctgcagtctggacctgagctggagaagcctggcgcttcagtgatgatatcctgcaaggcttctggttcctcattcactggctacaacatgaactgggtgaggcagaacattggaaagagccttgaatggattggagctattgatccttactatggtggaactagctacaaccagaagttcaagggcagggccacattgactgtagacaaatcgtccagcacagcctacatgcacctcaagagcctgacatctgaggactctgcagtctattactgtgtaagcggaatggagtactggggtcaaggaacctcagtcaccgtctcctcagcctccaccaagggcccatcggtcttccccctggcaccctcctccaagagcacctctgggggcacagcggccctgggctgcctggtcaaggactacttccccgaaccggtgacggtgtcgtggaactcaggcgccctgaccagcggcgtgcacaccttcccggctgtcctacagtcctcaggactctactccctcagcagcgtggtgaccgtgccctccagcagcttgggcacccagacctacatctgcaacgtgaatcacaagcccagcaacaccaaggtggacaagagagttgagcccaaatcttgtgacaaaactcacacatgcccaccgtgcccagcacctgaactcctggggggaccgtcagtcttcctcttccccccaaaacccaaggacaccctcatgatctcccggacccctgaggtcacatgcgtggtggtggacgtgagccacgaagaccctgaggtcaagttcaactggtacgtggacggcgtggaggtgcataatgccaagacaaagccgcgggaggagcagtacaacagcacgtaccgtgtggtcagcgtcctcaccgtcctgcaccaggactggctgaatggcaaggagtacaagtgcaaggtctccaacaaagccctcccagcccccatcgagaaaaccatctccaaagccaaagggcagccccgagaaccacaggtgtacaccctgcccccatcccgggaggagatgaccaagaaccaggtcagcctgacctgcctggtcaaaggcttctatcccagcgacatcgccgtggagtgggagagcaatgggcagccggagaacaactacaagaccacgcctcccgtgctggactccgacggctccttcttcctctatagcaagctcaccgtggacaagagcaggtggcagcaggggaacgtcttctcatgctccgtgatgcatgaggctctgcacaaccactacacgcagaagagcctctccctgtccccgggtaaatga

SEQ ID NO: 3 - protein, 240 aa, synthetic construct
  REGION 1..240: note = artificial antibody chain
MEAPAQLLFLLLLWLPDTTGEIVMTQSPATLSVSPGERATLSCRSSQSLVHRNGNTYLHWYLQKPGQSPKLLIHKVSNRFSGVPDRFSGSGSGTDFTLKISRVEAEDLGVYFCSQSTHVPPLTFGAGTKLELKRTVAAPSVFIFPPSDEQLKSGTASVVCLLNNFYPREAKVQWKVDNALQSGNSQESVTEQDSKDSTYSLSSTLTLSKADYEKHKVYACEVTHQGLSSPVTKSFNRGEC

SEQ ID NO: 4 - protein, 462 aa, synthetic construct
  REGION 1..462: note = artificial antibody chain
MGWTWIFILILSVTTGVHSEVQLLQSGPELEKPGASVMISCKASGSSFTGYNMNWVRQNIGKSLEWIGAIDPYYGGTSYNQKFKGRATLTVDKSSSTAYMHLKSLTSEDSAVYYCVSGMEYWGQGTSVTVSSASTKGPSVFPLAPSSKSTSGGTAALGCLVKDYFPEPVTVSWNSGALTSGVHTFPAVLQSSGLYSLSSVVTVPSSSLGTQTYICNVNHKPSNTKVDKRVEPKSCDKTHTCPPCPAPELLGGPSVFLFPPKPKDTLMISRTPEVTCVVVDVSHEDPEVKFNWYVDGVEVHNAKTKPREEQYNSTYRVVSVLTVLHQDWLNGKEYKCKVSNKALPAPIEKTISKAKGQPREPQVYTLPPSREEMTKNQVSLTCLVKGFYPSDIAVEWESNGQPENNYKTTPPVLDSDGSFFLYSKLTVDKSRWQQGNVFSCSVMHEALHNHYTQKSLSLSPGK

SEQ ID NO: 5 - DNA, 720 bp, synthetic construct
  source 1..720: mol_type = other DNA
  misc_feature 1..720: note = artificial antibody chain
atgaagttgcctgttaggctgttggtgctgatgttctggattcctgcttccttaagcgacgtggtgatgacccagacccccctgtccctgcccgtgacccccggcgagcccgcctccatctcctgcagatctagtcagagtcttgtacaccgtaatggaaacacctatttacattggtacctgcagaagccaggccagtctccaaagctcctgattcacaaagtttccaaccgattttctggggtcccagacaggttcagtggcagtggatcagggacagatttcacactcaagatcagcagagtggaggctgaggatctgggagtttatttctgttctcaaagtacacatgttcctccgctcacgttcggtgctgggaccaagctggagctgaaacgaactgtggctgcaccatctgtcttcatcttcccgccatctgatgagcagttgaaatctggaactgcctctgttgtgtgcctgctgaataacttctatcccagagaggccaaagtacagtggaaggtggataacgccctccaatcgggtaactcccaggagagtgtcacagagcaggacagcaaggacagcacctacagcctcagcagcaccctgacgctgagcaaagcagactacgagaaacacaaagtctacgcctgcgaagtcacccatcagggcctgagctcgcccgtcacaaagagcttcaacaggggagagtgttag

SEQ ID NO: 6 - DNA, 1788 bp, synthetic construct
  source 1..1788: mol_type = other DNA
  misc_feature 1..1788: note = artificial antibody chain
atgaagttgcctgttaggctgttggtgctgatgttctggattcctgcttccttaagcgaggtgcagctggtgcagtccggcgccgaggtggagaagcccggcgcctccgtgaagatctcctgcaaggcctccggctcctccttcaccggctacaacatgaactgggtgcgccagaacatcggcaagtccctggagtggatcggcgccatcgacccctactacggcggcacctcctacaaccagaagttcaagggccgcgccaccctgaccgtggacaagtccacctccaccgcctacatgcacctgaagtccctgcgctccgaggacaccgccgtgtactactgcgtgtccggcatggagtactggggccagggcacctccgtgaccgtgtcctccgcctccaccaagggcccatcggtcttccccctggcaccctcctccaagagcacctctgggggcacagcggccctgggctgcctggtcaaggactacttccccgaaccggtgacggtgtcgtggaactcaggcgccctgaccagcggcgtgcacaccttcccggctgtcctacagtcctcaggactctactccctcagcagcgtggtgaccgtgccctccagcagcttgggcacccagacctacatctgcaacgtgaatcacaagcccagcaacaccaaggtggacaagagagttgagcccaaatcttgtgacaaaactcacacatgcccaccgtgcccagcacctgaactcctggggggaccgtcagtcttcctcttccccccaaaacccaaggacaccctcatgatctcccggacccctgaggtcacatgcgtggtggtggacgtgagccacgaagaccctgaggtcaagttcaactggtacgtggacggcgtggaggtgcataatgccaagacaaagccgcgggaggagcagtacaacagcacgtaccgtgtggtcagcgtcctcaccgtcctgcaccaggactggctgaatggcaaggagtacaagtgcaaggtctccaacaaagccctcccagcccccatcgagaaaaccatctccaaagccaaagggcagccccgagaaccacaggtgtacaccctgcccccatcccgggaggagatgaccaagaaccaggtcagcctgacctgcctggtcaaaggcttctatcccagcgacatcgccgtggagtgggagagcaatgggcagccggagaacaactacaagaccacgcctcccgtgctggactccgacggctccttcttcctctatagcaagctcaccgtggacaagagcaggtggcagcaggggaacgtcttctcatgctccgtgatgcatgaggctctgcacaaccactacacgcagaagagcctctccctgtccccgggtaaagccccaacttcaagttctacaaagaaaacacagctgcaactggagcatctcctgctggatctccagatgattctgaatggaattaacaactacaagaatcccaaactcaccaggatgctcacattcaagttctacatgcccaagaaggccacagagctcaaacatctccagtgtctagaggaggaactcaaacctctggaggaagtgctaaacctcgctcagagcaaaaacttccacttaagacctagggacttaatcagcaatatcaacgtaatagttctggaactaaagggatccgaaacaacattcatgtgtgaatatgctgatgagacagcaaccattgtagaatttctgaacagatggattaccttttgtcaaagcatcatctcaacactaacttga

SEQ ID NO: 7 - protein, 239 aa, synthetic construct
  REGION 1..239: note = artificial antibody chain
MKLPVRLLVLMFWIPASLSDVVMTQTPLSLPVTPGEPASISCRSSQSLVHRNGNTYLHWYLQKPGQSPKLLIHKVSNRFSGVPDRFSGSGSGTDFTLKISRVEAEDLGVYFCSQSTHVPPLTFGAGTKLELKRTVAAPSVFIFPPSDEQLKSGTASVVCLLNNFYPREAKVQWKVDNALQSGNSQESVTEQDSKDSTYSLSSTLTLSKADYEKHKVYACEVTHQGLSSPVTKSFNRGEC

SEQ ID NO: 8 - protein, 595 aa, synthetic construct
  REGION 1..595: note = artificial antibody chain
MKLPVRLLVLMFWIPASLSEVQLVQSGAEVEKPGASVKISCKASGSSFTGYNMNWVRQNIGKSLEWIGAIDPYYGGTSYNQKFKGRATLTVDKSTSTAYMHLKSLRSEDTAVYYCVSGMEYWGQGTSVTVSSASTKGPSVFPLAPSSKSTSGGTAALGCLVKDYFPEPVTVSWNSGALTSGVHTFPAVLQSSGLYSLSSVVTVPSSSLGTQTYICNVNHKPSNTKVDKRVEPKSCDKTHTCPPCPAPELLGGPSVFLFPPKPKDTLMISRTPEVTCVVVDVSHEDPEVKFNWYVDGVEVHNAKTKPREEQYNSTYRVVSVLTVLHQDWLNGKEYKCKVSNKALPAPIEKTISKAKGQPREPQVYTLPPSREEMTKNQVSLTCLVKGFYPSDIAVEWESNGQPENNYKTTPPVLDSDGSFFLYSKLTVDKSRWQQGNVFSCSVMHEALHNHYTQKSLSLSPGKAPTSSSTKKTQLQLEHLLLDLQMILNGINNYKNPKLTRMLTFKFYMPKKATELKHLQCLEEELKPLEEVLNLAQSKNFHLRPRDLISNINVIVLELKGSETTFMCEYADETATIVEFLNRWITFCQSIISTLT